European Patent Application EP 4 613 857 A1, published September 10, 2025. Title: Amidase mutant and use thereof. Applicant: ASYMCHEM LIFE SCIENCE(TIANJIN) CO., LTD. The sequence listing filed with the application follows.

SEQUENCE LISTING (1 sequence)

SEQ ID NO: 1 - protein, 329 aa, Yersinia frederiksenii
MKWLEESIMVKRGVGAGRKPVTHHLTEEMQKEFHYTIGPYSTPVLTIEPGDRVIVDTRDAFEGAINSEQDIPSQLLKMPFLNPQNGPIMVNGAEKGDVIAVYIESMLPRGVNPHGICAMIPHFGGLTGTDLTAMLNDPLPEKVRMIKLDSEKVYWSERHTLPYKPHIGTLSVSPEIDSINSLTPDNHGGNMDVPDIGPGSITYLPVRAPGGRLFIGDAHACQGDGEICGTAVEFASITTIKVDLIKNWQLSWPRMENAETIMSIGSARPLEDATRIAYRDLIYWLVADFGFDQWDAYMLLSQCGKVRLGNMVDPKYTVGAMLNKELLAP